European Patent Application EP 4 310 176 A1, published January 24, 2024. Title: Pericytes transfected with the basic fibroblast growth factor (bFGF) gene. Applicant: Astellas Pharma Inc. Osaka University. The sequence listing filed with the application follows.

SEQUENCE LISTING (5 sequences)

SEQ ID NO: 1 - DNA, 3877 bp, Homo sapiens
  ref <308>: Genbank/M27968.1
  ref <309>: 1994-11-08
  ref <313>: (1)..(3877)
gccagattagcggacgcgtgcccgcggttgcaacgggatcccgggcgctgcagcttgggaggcggctctccccaggcggcgtccgcggagacaaccatccgtgaaccccaggtcccggcgcgccggctcgccgcgcaccaggggccggcggacagaagagcggccgagcggctcgaggctgggggacccggcgcggccgcgcgctgccgggcgggaggctggggggccggggcggggccgtgccccggagcgggtcggaggccggggccggggccgggggacggcggctccccgcgcggctccagcggctcggggatcccggccgggccccgcaggaccatggcagccgggagcatcaccacgctgcccgccttgcccgaggatggcggcagcggcgccttcccgcccggccacttcaaggaccccaagcggctgtactgcaaaaacgggggcttcttcctgcgcatccaccccgacggccgagttgacggggtccgggagaagagcgaccctcacatcaagctacaacttcaagcagaagagagaggagttgtgtctatcaaaggagtgtgtgctaaccgttacctggctatgaaggaagatggaagattactggcttctaaatgtgttacggatgagtgtttcttttttgaacgattggaatctaataactacaatacttaccggtcaaggaaatacaccagttggtatgtggcactgaaacgaactgggcagtataaacttggatccaaaacaggacctgggcagaaagctatactttttcttccaatgtctgctaagagctgattttaatggccacatctaatctcatttcacatgaaagaagaagtatattttagaaatttgttaatgagagtaaaagaaaataaatgtgtaaagctcagtttggataattggtcaaacaattttttatccagtagtaaaatatgtaaccattgtcccagtaaagaaaaataacaaaagttgtaaaatgtatattctcccttttatattgcatctgctgttacccagtgaagcttacctagagcaatgatctttttcacgcatttgctttattcgaaaagaggcttttaaaatgtgcatgtttagaaacaaaatttcttcatggaaatcatcatatacattagaaaatcacagtcagatgtttaatcaatccaaaatgtccactatttcttatgtcattcgttagtctacatgtttctaaacatataaatgtgaatttaatcaattcctttcatagttttataattctctggcagttccttatgatagagtttataaaacagtcctgtgtaaactgctggaagttcttccacagtcaggtcaattttgtcaaacccttctctgtacccatacagcagcagcctagcaactctgctggtgatgggagttgtattttcagtcttcgccaggtcattgagatccatccactcacatcttaagcattcttcctggcaaaaatttatggtgaatgaatatggctttaggcggcagatgatatacatatctgacttcccaaaagctccaggatttgtgtgctgttgccgaatactcaggacggacctgaattctgattttataccagtctcttcaaaaccttctcgaaccgctgtgtctcctacgtaaaaaaagagatgtacaaatcaataataattacacttttagaaactgtatcatcaaagattttcagttaaagtagcattatgtaaaggctcaaaacattaccctaacaaagtaaagttttcaatacaaattctttgccttgtggatatcaagaaatcccaaaatattttcttaccactgtaaattcaagaagcttttgaaatgctgaatatttctttggctgctacttggaggcttatctacctgtacatttttggggtcagctctttttaacttcttgctgctgtttttcccaaaaggtaaaaatatagattgaaaagttaaaacattttgcatggctgcagttcctttgtttcttgagataagattccaaagaacttagatttatttcttcaacaccgaaatgctggaggtgtttgatcagttttcaagaaacttggaatataaataattttataattcaacaaaggttttcacattttataaggttgatttttcaattaaatgcaaatttatgtggcaggatttttattgccattaacatatttttgtggctgctttttctacacatccagatggtccctctaactgggctttctctaattttgtgatgttctgtcattgtctcccaaagtatttaggagaagccctttaaaaagctgccttcctctaccactttgctgaaagcttcacaattgtcacagacaaagatttttgttccaatactcgttttgcctctattttacttgtttgtcaaatagtaaatgatatttgcccttgcagtaattctactggtgaaaaacatgcaaagaagaggaagtcacagaaacatgtctcaattcccatgtgctgtgactgtagactgtcttaccatagactgtcttacccatcccctggatatgctcttgttttttccctctaatagctatggaaagatgcatagaaagagtataatgttttaaaacataaggcattcgtctgccatttttcaattacatgctgacttcccttacaattgagatttgcccataggttaaacatggttagaaacaactgaaagcataaaagaaaaatctaggccgggtgcagtggctcatgcccatattccctgcactttgggaggccaaagcaggaggatcgcttgagcccaggagttcaagaccaacctggtgaaaccccgtctctacaaaaaaacacaaaaaatagccaggcatggtggcgtgtacatgtggtctcagatacttgggaggctgaggtgggagggttgatcacttgaggctgagaggtcaaggttacagtgagccataatcgtgccactgcagtccagcctaggcaacagagtgagactttgtctcaaaaaaagagaaattttccttaataagaaaagtaatttttactctgatgtgcaatacatttgttattaaatttattatttaagatggtagcactagtcttaaattgtataaaatatcccctaacatgtttaaatgtccatttttattcattatgctttgaaaaataattatggggaaatacatgtttgttattaaatttattattaaagatagtagcactagtcttaaatttgatataacatctcctaacttgtttaaatgtccatttttattctttatgtttgaaaataaattatggggatcctatttagctcttagtaccactaatcaaaagttcggcatgtagctcatgatctatgctgtttctatgtcgtggaagcaccggatgggggtagtgagcaaatctgccctgctcagcagtcaccatagcagctgactgaaaatcagcactgcctgagtagttttgatcagtttaacttgaatcactaactgactgaaaattgaatgggcaaataagtgcttttgtctccagagtatgcgggagacccttccacctcaagatggatatttcttccccaaggatttcaagatgaattgaaatttttaatcaagatagtgtgctttattctgttgtattttttattattttaatatactgtaagccaaactgaaataacatttgctgttttataggtttgaagacataggaaaaactaagaggttttatttttgtttttgctgatgaagagatatgtttaaatactgttgtattgttttgtttagttacaggacaataatgaaatggagtttatatttgttatttctattttgttatatttaataatagaattagattgaaataaaatataatgggaaat

SEQ ID NO: 2 - protein, 155 aa, Homo sapiens [sequence omitted]

SEQ ID NO: 3 - DNA, 1314 bp, Artificial Sequence
  nucleotide sequence of human bFGF analog
atggtggccggcacaagatgtctgctggccctgctgctgcctcaggtgctgctgggcggagctgctggactggtgcctgagctgggcagaagaaagttcgccgctgccagctccggcagacctagcagccagccttctgacgaggtgctgagcgagttcgagctgcggctgctgagcatgttcggcctgaagcagaggcccacccccagcagagatgctgtggtgcccccctacatgctggacctgtacagaaggcacagcggccagcctggaagccctgcccctgatcacagactggaaagagccgccagccgggccaataccgtgcggagctttcaccacgaggaatccctggaagaactgcccgagacaagcggcaagaccacccggcggttctttttcaacctgtcctccatccccaccgaagagttcatcaccagcgccgagctgcaggtgttccgcgagcagatgcaggatgccctgggcaacaacagcagcttccaccaccggatcaacatctacgagatcatcaagcccgccaccgccaacagcaagttccccgtgaccagactgctggacacccggctcgtgaaccagaacgccagcagatgggagagcttcgacgtgacccctgccgtgatgagatggacagcccagggccacgccaaccacggctttgtggtggaagtggcccacctggaagagaagcagggcgtgtccaagcggcacgtgcggatcagcagaagcctgcaccaggacgagcacagctggtcccagatcagacccctgctcgtgaccttcggccacgatggaagaggccacgccctgaccagaagaagaagggccaaaagggccgctggcagcatcaccacactgcctgccctgcctgaggatggcggatctggcgcttttccacccggccacttcaaggaccccaagcggctgtactgcaagaacggcggattcttcctgagaatccaccccgacggcagagtggacggcgtgcgggaaaagagcgacccccacatcaagctgcagctgcaggccgaagaacggggcgtggtgtctatcaaaggcgtgtccgccaatagatacctggccatgaaggaagatggccggctgctggcctccaagaacgtgaccgacgagtgcttcttctttgaacggctggaaagcaacaactacaacacctacagaagccggaagtacacctcttggtacgtggcactgaagcggaccggccagtacaagctgggctctaagacaggcccaggccagaaggccatcctgtttctgcccatgagcgccaagagc

SEQ ID NO: 4 - protein, 438 aa, Artificial Sequence
  amino acid sequence of human bFGF analog
MVAGTRCLLALLLPQVLLGGAAGLVPELGRRKFAAASSGRPSSQPSDEVLSEFELRLLSMFGLKQRPTPSRDAVVPPYMLDLYRRHSGQPGSPAPDHRLERAASRANTVRSFHHEESLEELPETSGKTTRRFFFNLSSIPTEEFITSAELQVFREQMQDALGNNSSFHHRINIYEIIKPATANSKFPVTRLLDTRLVNQNASRWESFDVTPAVMRWTAQGHANHGFVVEVAHLEEKQGVSKRHVRISRSLHQDEHSWSQIRPLLVTFGHDGRGHALTRRRRAKRAAGSITTLPALPEDGGSGAFPPGHFKDPKRLYCKNGGFFLRIHPDGRVDGVREKSDPHIKLQLQAEERGVVSIKGVSANRYLAMKEDGRLLASKNVTDECFFFERLESNNYNTYRSRKYTSWYVALKRTGQYKLGSKTGPGQKAILFLPMSAKS

SEQ ID NO: 5 - DNA, 8286 bp, Artificial Sequence
  nucleotide sequence of pLe6-Bmp-bFGF
aatgtagtcttatgcaatactcttgtagtcttgcaacatggtaacgatgagttagcaacatgccttacaaggagagaaaaagcaccgtgcatgccgattggtggaagtaaggtggtacgatcgtgccttattaggaaggcaacagacgggtctgacatggattggacgaaccactgaattgccgcattgcagagatattgtatttaagtgcctagctcgatacataaacgggtctctctggttagaccagatctgagcctgggagctctctggctaactagggaacccactgcttaagcctcaataaagcttgccttgagtgcttcaagtagtgtgtgcccgtctgttgtgtgactctggtaactagagatccctcagacccttttagtcagtgtggaaaatctctagcagtggcgcccgaacagggacttgaaagcgaaagggaaaccagaggagctctctcgacgcaggactcggcttgctgaagcgcgcacggcaagaggcgaggggcggcgactggtgagtacgccaaaaattttgactagcggaggctagaaggagagagatgggtgcgagagcgtcagtattaagcgggggagaattagatcgcgatgggaaaaaattcggttaaggccagggggaaagaaaaaatataaattaaaacatatagtatgggcaagcagggagctagaacgattcgcagttaatcctggcctgttagaaacatcagaaggctgtagacaaatactgggacagctacaaccatcccttcagacaggatcagaagaacttagatcattatataatacagtagcaaccctctattgtgtgcatcaaaggatagagataaaagacaccaaggaagctttagacaagatagaggaagagcaaaacaaaagtaagaccaccgcacagcaagcggccgctgatcttcagacctggaggaggagatatgagggacaattggagaagtgaattatataaatataaagtagtaaaaattgaaccattaggagtagcacccaccaaggcaaagagaagagtggtgcagagagaaaaaagagcagtgggaataggagctttgttccttgggttcttgggagcagcaggaagcactatgggcgcagcgtcaatgacgctgacggtacaggccagacaattattgtctggtatagtgcagcagcagaacaatttgctgagggctattgaggcgcaacagcatctgttgcaactcacagtctggggcatcaagcagctccaggcaagaatcctggctgtggaaagatacctaaaggatcaacagctcctggggatttggggttgctctggaaaactcatttgcaccactgctgtgccttggaatgctagttggagtaataaatctctggaacagatttggaatcacacgacctggatggagtgggacagagaaattaacaattacacaagcttaatacactccttaattgaagaatcgcaaaaccagcaagaaaagaatgaacaagaattattggaattagataaatgggcaagtttgtggaattggtttaacataacaaattggctgtggtatataaaattattcataatgatagtaggaggcttggtaggtttaagaatagtttttgctgtactttctatagtgaatagagttaggcagggatattcaccattatcgtttcagacccacctcccaaccccgaggggacccgacaggcccgaaggaatagaagaagaaggtggagagagagacagagacagatccattcgattagtgaacggatctcgacggtatcgataagcttgggagttccgcgttacataacttacggtaaatggcccgcctggctgaccgcccaacgacccccgcccattgacgtcaataatgacgtatgttcccatagtaacgccaatagggactttccattgacgtcaatgggtggagtatttacggtaaactgcccacttggcagtacatcaagtgtatcatatgccaagtacgccccctattgacgtcaatgacggtaaatggcccgcctggcattatgcccagtacatgaccttatgggactttcctacttggcagtacatctacgtattagtcatcgctattaccatggtgatgcggttttggcagtacatcaatgggcgtggatagcggtttgactcacggggatttccaagtctccaccccattgacgtcaatgggagtttgttttggcaccaaaatcaacgggactttccaaaatgtcgtaacaactccgccccattgacgcaaatgggcggtaggcgtgtacggtgggaggtctatataagcagagctcgtttagtgaaccgtcagatcgcctggagacgccatccacgctgttttgacctccatagaagacaccgactctagaggatccactagtccagtgtggtggaattgatcccttcaccgccaccatggtggccggcacaagatgtctgctggccctgctgctgcctcaggtgctgctgggcggagctgctggactggtgcctgagctgggcagaagaaagttcgccgctgccagctccggcagacctagcagccagccttctgacgaggtgctgagcgagttcgagctgcggctgctgagcatgttcggcctgaagcagaggcccacccccagcagagatgctgtggtgcccccctacatgctggacctgtacagaaggcacagcggccagcctggaagccctgcccctgatcacagactggaaagagccgccagccgggccaataccgtgcggagctttcaccacgaggaatccctggaagaactgcccgagacaagcggcaagaccacccggcggttctttttcaacctgtcctccatccccaccgaagagttcatcaccagcgccgagctgcaggtgttccgcgagcagatgcaggatgccctgggcaacaacagcagcttccaccaccggatcaacatctacgagatcatcaagcccgccaccgccaacagcaagttccccgtgaccagactgctggacacccggctcgtgaaccagaacgccagcagatgggagagcttcgacgtgacccctgccgtgatgagatggacagcccagggccacgccaaccacggctttgtggtggaagtggcccacctggaagagaagcagggcgtgtccaagcggcacgtgcggatcagcagaagcctgcaccaggacgagcacagctggtcccagatcagacccctgctcgtgaccttcggccacgatggaagaggccacgccctgaccagaagaagaagggccaaaagggccgctggcagcatcaccacactgcctgccctgcctgaggatggcggatctggcgcttttccacccggccacttcaaggaccccaagcggctgtactgcaagaacggcggattcttcctgagaatccaccccgacggcagagtggacggcgtgcgggaaaagagcgacccccacatcaagctgcagctgcaggccgaagaacggggcgtggtgtctatcaaaggcgtgtccgccaatagatacctggccatgaaggaagatggccggctgctggcctccaagaacgtgaccgacgagtgcttcttctttgaacggctggaaagcaacaactacaacacctacagaagccggaagtacacctcttggtacgtggcactgaagcggaccggccagtacaagctgggctctaagacaggcccaggccagaaggccatcctgtttctgcccatgagcgccaagagctgaaagggctcgagtctagagggcccgcggttcgaaggtaagcctatccctaaccctctcctcggtctcgattctacgcgtaccggttagtaatgagtttggaattaattctgtggaatgtgtgtcagttagggtgtggaaagtccccaggctccccagcaggcagaagtatgcaaagcatgcatctcaattagtcagcaaccaggtgtggaaagtccccaggctccccagcaggcagaagtatgcaaagcatgcatctcaattagtcagcaaccatagtcccgcccctaactccgcccatcccgcccctaactccgcccagttccgcccattctccgccccatggctgactaattttttttatttatgcagaggccgaggccgcctctgcctctgagctattccagaagtagtgaggaggcttttttggaggcctaggcttttgcaaaaagctcccgggagcttgtatatccattttcggatctgatcagcacgtgttgacaattaatcatcggcatagtatatcggcatagtataatacgacaaggtgaggaactaaaccatggccaagcctttgtctcaagaagaatccaccctcattgaaagagcaacggctacaatcaacagcatccccatctctgaagactacagcgtcgccagcgcagctctctctagcgacggccgcatcttcactggtgtcaatgtatatcattttactgggggaccttgtgcagaactcgtggtgctgggcactgctgctgctgcggcagctggcaacctgacttgtatcgtcgcgatcggaaatgagaacaggggcatcttgagcccctgcggacggtgccgacaggtgcttctcgatctgcatcctgggatcaaagccatagtgaaggacagtgatggacagccgacggcagttgggattcgtgaattgctgccctctggttatgtgtgggagggctaagcacaattcgagctcggtacctttaagaccaatgacttacaaggcagctgtagatcttagccactttttaaaagaaaaggggggactggaagggctaattcactcccaacgaagacaagatctgctttttgcttgtactgggtctctctggttagaccagatctgagcctgggagctctctggctaactagggaacccactgcttaagcctcaataaagcttgccttgagtgcttcaagtagtgtgtgcccgtctgttgtgtgactctggtaactagagatccctcagacccttttagtcagtgtggaaaatctctagcagtagtagttcatgtcatcttattattcagtatttataacttgcaaagaaatgaatatcagagagtgagaggaacttgtttattgcagcttataatggttacaaataaagcaatagcatcacaaatttcacaaataaagcatttttttcactgcattctagttgtggtttgtccaaactcatcaatgtatcttatcatgtctggctctagctatcccgcccctaactccgcccatcccgcccctaactccgcccagttccgcccattctccgccccatggctgactaattttttttatttatgcagaggccgaggccgcctcggcctctgagctattccagaagtagtgaggaggcttttttggaggcctagggacgtacccaattcgccctatagtgagtcgtattacgcgcgctcactggccgtcgttttacaacgtcgtgactgggaaaaccctggcgttacccaacttaatcgccttgcagcacatccccctttcgccagctggcgtaatagcgaagaggcccgcaccgatcgcccttcccaacagttgcgcagcctgaatggcgaatgggacgcgccctgtagcggcgcattaagcgcggcgggtgtggtggttacgcgcagcgtgaccgctacacttgccagcgccctagcgcccgctcctttcgctttcttcccttcctttctcgccacgttcgccggctttccccgtcaagctctaaatcgggggctccctttagggttccgatttagtgctttacggcacctcgaccccaaaaaacttgattagggtgatggttcacgtagtgggccatcgccctgatagacggtttttcgccctttgacgttggagtccacgttctttaatagtggactcttgttccaaactggaacaacactcaaccctatctcggtctattcttttgatttataagggattttgccgatttcggcctattggttaaaaaatgagctgatttaacaaaaatttaacgcgaattttaacaaaatattaacgcttacaatttaggtggcacttttcggggaaatgtgcgcggaacccctatttgtttatttttctaaatacattcaaatatgtatccgctcatgagacaataaccctgataaatgcttcaataatattgaaaaaggaagagtatgagtattcaacatttccgtgtcgcccttattcccttttttgcggcattttgccttcctgtttttgctcacccagaaacgctggtgaaagtaaaagatgctgaagatcagttgggtgcacgagtgggttacatcgaactggatctcaacagcggtaagatccttgagagttttcgccccgaagaacgttttccaatgatgagcacttttaaagttctgctatgtggcgcggtattatcccgtattgacgccgggcaagagcaactcggtcgccgcatacactattctcagaatgacttggttgagtactcaccagtcacagaaaagcatcttacggatggcatgacagtaagagaattatgcagtgctgccataaccatgagtgataacactgcggccaacttacttctgacaacgatcggaggaccgaaggagctaaccgcttttttgcacaacatgggggatcatgtaactcgccttgatcgttgggaaccggagctgaatgaagccataccaaacgacgagcgtgacaccacgatgcctgtagcaatggcaacaacgttgcgcaaactattaactggcgaactacttactctagcttcccggcaacaattaatagactggatggaggcggataaagttgcaggaccacttctgcgctcggcccttccggctggctggtttattgctgataaatctggagccggtgagcgtgggtctcgcggtatcattgcagcactggggccagatggtaagccctcccgtatcgtagttatctacacgacggggagtcaggcaactatggatgaacgaaatagacagatcgctgagataggtgcctcactgattaagcattggtaactgtcagaccaagtttactcatatatactttagattgatttaaaacttcatttttaatttaaaaggatctaggtgaagatcctttttgataatctcatgaccaaaatcccttaacgtgagttttcgttccactgagcgtcagaccccgtagaaaagatcaaaggatcttcttgagatcctttttttctgcgcgtaatctgctgcttgcaaacaaaaaaaccaccgctaccagcggtggtttgtttgccggatcaagagctaccaactctttttccgaaggtaactggcttcagcagagcgcagataccaaatactgttcttctagtgtagccgtagttaggccaccacttcaagaactctgtagcaccgcctacatacctcgctctgctaatcctgttaccagtggctgctgccagtggcgataagtcgtgtcttaccgggttggactcaagacgatagttaccggataaggcgcagcggtcgggctgaacggggggttcgtgcacacagcccagcttggagcgaacgacctacaccgaactgagatacctacagcgtgagctatgagaaagcgccacgcttcccgaagggagaaaggcggacaggtatccggtaagcggcagggtcggaacaggagagcgcacgagggagcttccagggggaaacgcctggtatctttatagtcctgtcgggtttcgccacctctgacttgagcgtcgatttttgtgatgctcgtcaggggggcggagcctatggaaaaacgccagcaacgcggcctttttacggttcctggccttttgctggccttttgctcacatgttctttcctgcgttatcccctgattctgtggataaccgtattaccgcctttgagtgagctgataccgctcgccgcagccgaacgaccgagcgcagcgagtcagtgagcgaggaagcggaagagcgcccaatacgcaaaccgcctctccccgcgcgttggccgattcattaatgcagctggcacgacaggtttcccgactggaaagcgggcagtgagcgcaacgcaattaatgtgagttagctcactcattaggcaccccaggctttacactttatgcttccggctcgtatgttgtgtggaattgtgagcggataacaatttcacacaggaaacagctatgaccatgattacgccaagcgcgcaattaaccctcactaaagggaacaaaagctggagctgcaagctt